European Patent Specification EP 3 433 257 B1, published October 11, 2023. Title: ALKYNYL NUCLEOSIDE ANALOGS AS INHIBITORS OF HUMAN RHINOVIRUS. Applicant: Novartis AG. Application PCT/IB2017/051638. The sequence listing filed with the application follows.

SEQUENCE LISTING (2 sequences)

SEQ ID NO: 1 - DNA, 22 bp, synthetic
ttttgtctttgtactaggaggc

SEQ ID NO: 2 - RNA, 12 nt, synthetic
uuuugccgcgcc